European Patent Application EP 4 163 290 A1, published April 12, 2023. Title: IMMUNOGENS FOR HIV VACCINATION. Applicant: FUNDACIO PRIVADA INSTITUT DE RECERCA DE LA SIDA - CAIXA. The sequence listing filed with the application follows.

SEQUENCE LISTING (98 sequences)

SEQ ID NO: 1 - protein, 78 aa, synthetic construct
  REGION 1..78: note = OLP HIV clade B consensus sequence
EKIRLRPGGKKKYKLKHIVWASRELERFAVNPGLLETSEGCRQILGQLQPSLQTGSEELKSLYNTVATLYCVHQKIEV

SEQ ID NO: 2 - protein, 14 aa, synthetic construct
  REGION 1..14: note = OLP HIV clade B consensus sequence
KAFSPEVIPMFSAL

SEQ ID NO: 3 - protein, 11 aa, synthetic construct
  REGION 1..11: note = OLP HIV clade B consensus sequence
GHQAAMQMLKE

SEQ ID NO: 4 - protein, 60 aa, synthetic construct
  REGION 1..60: note = OLP HIV clade B consensus sequence
IAPGQMREPRGSDIAGTTSTLQEQIGWMTNNPPIPVGEIYKRWIILGLNKIVRMYSPTSI

SEQ ID NO: 5 - protein, 14 aa, synthetic construct
  REGION 1..14: note = OLP HIV clade B consensus sequence
YVDRFYKTLRAEQA

SEQ ID NO: 6 - protein, 15 aa, synthetic construct
  REGION 1..15: note = OLP HIV clade B consensus sequence
ACQGVGGPGHKARVL

SEQ ID NO: 7 - protein, 27 aa, synthetic construct
  REGION 1..27: note = OLP HIV clade B consensus sequence
CTERQANFLGKIWPSHKGRPGNFLQSR

SEQ ID NO: 8 - protein, 55 aa, synthetic construct
  REGION 1..55: note = OLP HIV clade B consensus sequence
KMIGGIGGFIKVRQYDQILIEICGHKAIGTVLVGPTPVNIIGRNLLTQIGCTLNF

SEQ ID NO: 9 - protein, 17 aa, synthetic construct
  REGION 1..17: note = OLP HIV clade B consensus sequence
LVEICTELEKEGKISKI

SEQ ID NO: 10 - protein, 55 aa, synthetic construct
  REGION 1..55: note = OLP HIV clade B consensus sequence
LRWGFTTPDKKHQKEPPFLWMGYELHPDKWTVQPIVLPEKDSWTVNDIQKLVGKL

SEQ ID NO: 11 - protein, 34 aa, synthetic construct
  REGION 1..34: note = OLP HIV clade B consensus sequence
ILKEPVHGVYYDPSKDLIAEIQKQGQGQWTYQIY

SEQ ID NO: 12 - protein, 34 aa, synthetic construct
  REGION 1..34: note = OLP HIV clade B consensus sequence
TKELQKQITKIQNFRVYYRDSRDPLWKGPAKLLW

SEQ ID NO: 13 - protein, 17 aa, synthetic construct
  REGION 1..17: note = OLP HIV clade B consensus sequence
KIIRDYGKQMAGDDCVA

SEQ ID NO: 14 - protein, 26 aa, synthetic construct
  REGION 1..26: note = OLP HIV clade B consensus sequence
VKHHMYISKKAKGWFYRHHYESTHPR

SEQ ID NO: 15 - protein, 19 aa, synthetic construct
  REGION 1..19: note = OLP HIV clade B consensus sequence
VTKLTEDRWNKPQKTKGHR

SEQ ID NO: 16 - protein, 13 aa, synthetic construct
  REGION 1..13: note = OLP HIV clade B consensus sequence
AWLEAQEEEEVGF

SEQ ID NO: 17 - protein, 23 aa, synthetic construct
  REGION 1..23: note = OLP HIV clade B consensus sequence
EKIRLRPGGKKKYKLKHIVWASR

SEQ ID NO: 18 - protein, 22 aa, synthetic construct
  REGION 1..22: note = OLP HIV clade B consensus sequence
KLKHIVWASRELERFAVNPGLL

SEQ ID NO: 19 - protein, 23 aa, synthetic construct
  REGION 1..23: note = OLP HIV clade B consensus sequence
ERFAVNPGLLETSEGCRQILGQL

SEQ ID NO: 20 - protein, 24 aa, synthetic construct
  REGION 1..24: note = OLP HIV clade B consensus sequence
EGCRQILGQLQPSLQTGSEELKSL

SEQ ID NO: 21 - protein, 26 aa, synthetic construct
  REGION 1..26: note = OLP HIV clade B consensus sequence
QTGSEELKSLYNTVATLYCVHQRIEV

SEQ ID NO: 22 - protein, 14 aa, synthetic construct
  REGION 1..14: note = OLP HIV clade B consensus sequence
KAFSPEVIPMFSAL

SEQ ID NO: 23 - protein, 11 aa, synthetic construct
  REGION 1..11: note = OLP HIV clade B consensus sequence
GHQAAMQMLKE

SEQ ID NO: 24 - protein, 21 aa, synthetic construct
  REGION 1..21: note = OLP HIV clade B consensus sequence
IAPGQMREPRGSDIAGTTSTL

SEQ ID NO: 25 - protein, 23 aa, synthetic construct
  REGION 1..23: note = OLP HIV clade B consensus sequence
SDIAGTTSTLQEQIGWMTNNPPI

SEQ ID NO: 26 - protein, 24 aa, synthetic construct
  REGION 1..24: note = OLP HIV clade B consensus sequence
IGWMTNNPPIPVGEIYKRWIILGL

SEQ ID NO: 27 - protein, 22 aa, synthetic construct
  REGION 1..22: note = OLP HIV clade B consensus sequence
IYKRWIILGLNKIVRMYSPTSI

SEQ ID NO: 28 - protein, 14 aa, synthetic construct
  REGION 1..14: note = OLP HIV clade B consensus sequence
YVDRFYKTLRAEQA

SEQ ID NO: 29 - protein, 15 aa, synthetic construct
  REGION 1..15: note = OLP HIV clade B consensus sequence
ACQGVGGPGHKARVL

SEQ ID NO: 30 - protein, 27 aa, synthetic construct
  REGION 1..27: note = OLP HIV clade B consensus sequence
CTERQANFLGKIWPSHKGRPGNFLQSR

SEQ ID NO: 31 - protein, 26 aa, synthetic construct
  REGION 1..26: note = OLP HIV clade B consensus sequence
KMIGGIGGFIKVRQYDQILIEICGHK

SEQ ID NO: 32 - protein, 24 aa, synthetic construct
  REGION 1..24: note = OLP HIV clade B consensus sequence
QILIEICGHKAIGTVLVGPTPVNI

SEQ ID NO: 33 - protein, 25 aa, synthetic construct
  REGION 1..25: note = OLP HIV clade B consensus sequence
VLVGPTPVNIIGRNLLTQIGCTLNF

SEQ ID NO: 34 - protein, 17 aa, synthetic construct
  REGION 1..17: note = OLP HIV clade B consensus sequence
LVEICTEMEKEGKISKI

SEQ ID NO: 35 - protein, 25 aa, synthetic construct
  REGION 1..25: note = OLP HIV clade B consensus sequence
LRWGFTTPDKKHQKEPPFLWMGYEL

SEQ ID NO: 36 - protein, 25 aa, synthetic construct
  REGION 1..25: note = OLP HIV clade B consensus sequence
PPFLWMGYELHPDKWTVQPIVLPEK

SEQ ID NO: 37 - protein, 25 aa, synthetic construct
  REGION 1..25: note = OLP HIV clade B consensus sequence
TVQPIVLPEKDSWTVNDIQKLVGKL

SEQ ID NO: 38 - protein, 23 aa, synthetic construct
  REGION 1..23: note = OLP HIV clade B consensus sequence
ILKEPVHGVYYDPSKDLIAEIQK

SEQ ID NO: 39 - protein, 21 aa, synthetic construct
  REGION 1..21: note = OLP HIV clade B consensus sequence
SKDLIAEIQKQGQGQWTYQIY

SEQ ID NO: 40 - protein, 22 aa, synthetic construct
  REGION 1..22: note = OLP HIV clade B consensus sequence
TKELQKQITKIQNFRVYYRDSR

SEQ ID NO: 41 - protein, 22 aa, synthetic construct
  REGION 1..22: note = OLP HIV clade B consensus sequence
NFRVYYRDSRDPLWKGPAKLLW

SEQ ID NO: 42 - protein, 17 aa, synthetic construct
  REGION 1..17: note = OLP HIV clade B consensus sequence
KIIRDYGKQMAGDDCVA

SEQ ID NO: 43 - protein, 26 aa, synthetic construct
  REGION 1..26: note = OLP HIV clade B consensus sequence
VKHHMYISKKAKGWFYRHHYESTHPR

SEQ ID NO: 44 - protein, 19 aa, synthetic construct
  REGION 1..19: note = OLP HIV clade B consensus sequence
VTKLTEDRWNKPQKTKGHR

SEQ ID NO: 45 - protein, 13 aa, synthetic construct
  REGION 1..13: note = OLP HIV clade B consensus sequence
AWLEAQEEEEVGF

SEQ ID NO: 46 - protein, 17 aa, Homo sapiens
MWLQSLLLLGTVACSIS

SEQ ID NO: 47 - protein, 18 aa, synthetic construct
  REGION 1..18: note = human GM-CSF signal peptide + V
MWLQSLLLLGTVACSISV

SEQ ID NO: 48 - protein, 9 aa, synthetic construct
  REGION 1..9: note = Flag-tag
DYKDDDDKL

SEQ ID NO: 49 - protein, 556 aa, synthetic construct
  REGION 1..556: note = HIV immunogen comprising OLPs
MWLQSLLLLGTVACSISVEKIRLRPGGKKKYKLKHIVWASRELERFAVNPGLLETSEGCRQILGQLQPSLQTGSEELKSLYNTVATLYCVHQKIEVAAAKAFSPEVIPMFSALAAAGHQAAMQMLKEAAAIAPGQMREPRGSDIAGTTSTLQEQIGWMTNNPPIPVGEIYKRWIILGLNKIVRMYSPTSIAAAYVDRFYKTLRAEQAAACQGVGGPGHKARVLAAACTERQANFLGKIWPSHKGRPGNFLQSRAAAKMIGGIGGFIKVRQYDQILIEICGHKAIGTVLVGPTPVNIIGRNLLTQIGCTLNFAALVEICTEMEKEGKISKIAAALRWGFTTPDKKHQKEPPFLWMGYELHPDKWTVQPIVLPEKDSWTVNDIQKLVGKLAAAILKEPVHGVYYDPSKDLIAEIQKQGQGQWTYQIYAAATKELQKQITKIQNFRVYYRDSRDPLWKGPAKLLWAAAKIIRDYGKQMAGDDCVAAAVKHHMYISKKAKGWFYRHHYESTHPRAAAVTKLTEDRWNKPQKTKGHRAAAWLEAQEEEEVGFDYKDDDDKL

SEQ ID NO: 50 - DNA, 1674 bp, synthetic construct
  misc_feature 1..1674: note = polynucleotide encoding immunogen comprising HIV OLPs
  source 1..1674: mol_type = other DNA
atgtggctccagagcctgctactcctggggacggtggcctgcagcatctcggtcgagaagatccggctgcggccaggcggaaagaagaagtacaagctgaagcacatcgtctgggcctcgagggagctggagcggttcgcggtgaacccgggacttctggagacgtcggaggggtgcaggcagatcctcggccagctgcagccctctctgcaaacggggtctgaggagctgaagagcctgtacaacacggtggcgaccctctactgcgtccaccagaagatcgaggtggcagcggccaaggcgttctcgccggaggtcatccccatgttctcggcgctggcagctgccggacaccaggccgcgatgcagatgctgaaggaggccgctgcgatcgcaccgggccagatgagggagccacgcggttccgacatcgcgggaaccacctcgacgctccaggagcagatcggatggatgacgaacaacccgccaatcccggtcggggagatctacaagcggtggatcatcctcgggctgaacaagatcgtccggatgtacagcccgacgtcgatcgctgcggcatacgttgaccggttctacaagaccctgagggccgagcaggcagcggcctgccagggggtcggtggaccagggcacaaggcccgagtgctcgcggccgcatgcacggagcggcaggcgaacttcctggggaagatctggccgtcgcacaagggccgaccgggaaacttcctccagtctcgcgcagcggctaagatgatcggaggcatcggaggcttcatcaaagtccgtcagtacgaccagatcctcatcgagatctgcgggcacaaggcgatcggaaccgtgctcgtcggcccaacgcccgtgaacatcatcggccgcaacctgttaacgcagatcggctgcaccctcaacttcgccgcactagtggagatctgcacggagatggagaaggagggcaagatatcgaagatcgcggcagctctgaggtggggcttcaccacgccggacaagaagcaccagaaggagccgccattcctgtggatgggatacgagctgcacccggacaagtggaccgtgcagcccatcgtcctgccggagaaggactcgtggacggtgaacgacatccagaagctcgtggggaagctggcggcagccatcctcaaggagcccgtccacggggtgtactacgacccctctaaggacctgatcgcggagatccagaagcaggggcagggtcagtggacctaccagatctacgcagcagcaaccaaggagctgcagaagcagatcacgaagatccagaacttccgcgtatactaccgcgactcgcgggaccccctgtggaagggccctgcgaagcttctctgggcagccgcgaagatcatccgggactacggcaagcagatggcgggcgacgactgcgtggccgcagcggtgaagcaccatatgtacatctcgaagaaggcgaagggctggttctacagacaccactacgagtccacccaccccagggcagctgcggtgacgaagctgacggaggaccggtggaacaagccccagaagacgaagggtcaccgggcggctgcatggctggaggctcaggaggaggaggaggtgggcttcgattacaaggacgatgacgacaagctgtgataa

SEQ ID NO: 51 - DNA, 60 bp, synthetic construct
  misc_feature 1..60: note = 198HPlus primer
  source 1..60: mol_type = other DNA
gtcaccgggcggctgcatggctggaggctcaggaggaggaggaggtgggcttctgataag

SEQ ID NO: 52 - DNA, 59 bp, synthetic construct
  misc_feature 1..59: note = 298HMinus primer
  source 1..59: mol_type = other DNA
aattcttatcagaagcccacctcctcctcctcctgagcctccagccatgcagccgcccg

SEQ ID NO: 53 - protein, 18 aa, synthetic construct
  REGION 1..18: note = OLP clade B consensus sequence
EKIRLRPGGKKKYKLKHI

SEQ ID NO: 54 - protein, 15 aa, synthetic construct
  REGION 1..15: note = OLP clade B consensus sequence
ASRELERFAVNPGLL

SEQ ID NO: 55 - protein, 17 aa, synthetic construct
  REGION 1..17: note = OLP clade B consensus sequence
ERFAVNPGLLETSEGCR

SEQ ID NO: 56 - protein, 17 aa, synthetic construct
  REGION 1..17: note = OLP clade B consensus sequence
QLQPSLQTGSEELRSLY

SEQ ID NO: 57 - protein, 18 aa, synthetic construct
  REGION 1..18: note = OLP clade B consensus sequence
SLYNTVATLYCVHQRIEV

SEQ ID NO: 58 - protein, 17 aa, synthetic construct
  REGION 1..17: note = OLP clade B consensus sequence
AFSPEVIPMFSALSEGA

SEQ ID NO: 59 - protein, 15 aa, synthetic construct
  REGION 1..15: note = OLP clade B consensus sequence
IAPGQMREPRGSDIA

SEQ ID NO: 60 - protein, 18 aa, synthetic construct
  REGION 1..18: note = OLP clade B consensus sequence
STLQEQIGWMTNNPPIPV

SEQ ID NO: 61 - protein, 18 aa, synthetic construct
  REGION 1..18: note = OLP clade B consensus sequence
ACQGVGGPGHKARVLAEA

SEQ ID NO: 62 - protein, 18 aa, synthetic construct
  REGION 1..18: note = OLP clade B consensus sequence
GKIWPSHKGRPGNFLQSR

SEQ ID NO: 63 - protein, 18 aa, synthetic construct
  REGION 1..18: note = OLP clade B consensus sequence
WLEAQEEEEVGFPVRPQV

SEQ ID NO: 64 - protein, 18 aa, synthetic construct
  REGION 1..18: note = OLP clade B consensus sequence
EVGFPVRPQVPLRPMTYK

SEQ ID NO: 65 - protein, 18 aa, synthetic construct
  REGION 1..18: note = OLP clade B consensus sequence
NYTPGPGIRYPLTFGWCF

SEQ ID NO: 66 - protein, 15 aa, synthetic construct
  REGION 1..15: note = OLP clade B consensus sequence
RYPLTFGWCFKLVPV

SEQ ID NO: 67 - protein, 17 aa, synthetic construct
  REGION 1..17: note = OLP clade B consensus sequence
SLHGMDDPEKEVLVWKF

SEQ ID NO: 68 - protein, 18 aa, synthetic construct
  REGION 1..18: note = OLP clade B consensus sequence
KMIGGIGGFIKVRQYDQI

SEQ ID NO: 69 - protein, 18 aa, synthetic construct
  REGION 1..18: note = OLP clade B consensus sequence
FIKVRQYDQILIEICGHK

SEQ ID NO: 70 - protein, 17 aa, synthetic construct
  REGION 1..17: note = OLP clade B consensus sequence
QILIEICGHKAIGTVLV

SEQ ID NO: 71 - protein, 18 aa, synthetic construct
  REGION 1..18: note = OLP clade B consensus sequence
LVGPTPVNIIGRNLLTQI

SEQ ID NO: 72 - protein, 17 aa, synthetic construct
  REGION 1..17: note = OLP clade B consensus sequence
LVEICTEMEKEGKISKI

SEQ ID NO: 73 - protein, 18 aa, synthetic construct
  REGION 1..18: note = OLP clade B consensus sequence
LDVGDAYFSVPLDKDFRK

SEQ ID NO: 74 - protein, 18 aa, synthetic construct
  REGION 1..18: note = OLP clade B consensus sequence
LRWGFTTPDKKHQKEPPF

SEQ ID NO: 75 - protein, 18 aa, synthetic construct
  REGION 1..18: note = OLP clade B consensus sequence
DKKHQKEPPFLWMGYELH

SEQ ID NO: 76 - protein, 15 aa, synthetic construct
  REGION 1..15: note = OLP clade B consensus sequence
EIQKQGQGQWTYQIY

SEQ ID NO: 77 - protein, 18 aa, synthetic construct
  REGION 1..18: note = OLP clade B consensus sequence
PPLVKLWYQLEKEPIVGA

SEQ ID NO: 78 - protein, 15 aa, synthetic construct
  REGION 1..15: note = OLP clade B consensus sequence
IHLALQDSGLEVNIV

SEQ ID NO: 79 - protein, 18 aa, synthetic construct
  REGION 1..18: note = OLP clade B consensus sequence
VYLAWVPAHKGIGGNEQV

SEQ ID NO: 80 - protein, 16 aa, synthetic construct
  REGION 1..16: note = OLP clade B consensus sequence
SAGIRKVLFLDGIDKA

SEQ ID NO: 81 - protein, 18 aa, synthetic construct
  REGION 1..18: note = OLP clade B consensus sequence
TKELQKQITKIQNFRVYY

SEQ ID NO: 82 - protein, 18 aa, synthetic construct
  REGION 1..18: note = OLP clade B consensus sequence
TKIQNFRVYYRDSRDPLW

SEQ ID NO: 83 - protein, 18 aa, synthetic construct
  REGION 1..18: note = OLP clade B consensus sequence
YYRDSRDPLWKGPAKLLW

SEQ ID NO: 84 - protein, 17 aa, synthetic construct
  REGION 1..17: note = OLP clade B consensus sequence
KIIRDYGKQMAGDDCVA

SEQ ID NO: 85 - protein, 18 aa, synthetic construct
  REGION 1..18: note = OLP clade B consensus sequence
GPQREPYNEWTLELLEEL

SEQ ID NO: 86 - protein, 18 aa, synthetic construct
  REGION 1..18: note = OLP clade B consensus sequence
DLNNNTNTTSSSGEKMEK

SEQ ID NO: 87 - protein, 18 aa, synthetic construct
  REGION 1..18: note = OLP clade B consensus sequence
IRDKVQKEYALFYKLDVV

SEQ ID NO: 88 - protein, 18 aa, synthetic construct
  REGION 1..18: note = OLP clade B consensus sequence
YRLISCNTSVITQACPKV

SEQ ID NO: 89 - protein, 18 aa, synthetic construct
  REGION 1..18: note = OLP clade B consensus sequence
SVITQACPKVSFEPIPIH

SEQ ID NO: 90 - protein, 16 aa, synthetic construct
  REGION 1..16: note = OLP clade B consensus sequence
TNVSTVQCTHGIRPVV

SEQ ID NO: 91 - protein, 18 aa, synthetic construct
  REGION 1..18: note = OLP clade B consensus sequence
VAPTKAKRRVVQREKRAV

SEQ ID NO: 92 - protein, 18 aa, synthetic construct
  REGION 1..18: note = OLP clade B consensus sequence
VIEVVQRACRAILHIPRR

SEQ ID NO: 93 - protein, 18 aa, synthetic construct
  REGION 1..18: note = OLP clade B consensus sequence
VKHHMYISGKAKGWFYRH

SEQ ID NO: 94 - protein, 18 aa, synthetic construct
  REGION 1..18: note = OLP clade B consensus sequence
GKAKGWFYRHHYESTHPR

SEQ ID NO: 95 - protein, 18 aa, synthetic construct
  REGION 1..18: note = OLP clade B consensus sequence
TKLTEDRWNKPQKTKGHR

SEQ ID NO: 96 - protein, 6 aa, synthetic construct
  REGION 1..6: note = Tag sequence
AHGHRP

SEQ ID NO: 97 - protein, 14 aa, synthetic construct
  REGION 1..14: note = Tag sequence
PIHDHDHPHLVIHS

SEQ ID NO: 98 - protein, 7 aa, synthetic construct
  REGION 1..7: note = Tag sequence
  REGION 5..6: note = MISC_FEATURE - Xaa can be any naturally occurring amino acid
GMTCXXC